European Patent Application EP 4 201 957 A1, published June 28, 2023. Title: Modified Antibody and Method of Producing the Same. Applicant: Pharmabcine Inc. The sequence listing filed with the application follows.

SEQUENCE LISTING (51 sequences)

SEQ ID NO: 1 - protein, 8 aa, Artificial Sequence
  HCDR1
GFSFDDYA

SEQ ID NO: 2 - protein, 8 aa, Artificial Sequence
  HCDR2
IKDDGSQT

SEQ ID NO: 3 - protein, 13 aa, Artificial Sequence
  HCDR3
TTEGLMNGLHFDM

SEQ ID NO: 4 - protein, 9 aa, Artificial Sequence
  LCDR1
SSNIGAGYD

SEQ ID NO: 5 - protein, 3 aa, Artificial Sequence
  LCDR2
GNN

SEQ ID NO: 6 - protein, 10 aa, Artificial Sequence
  LCDR3
QSYDSRLGVV

SEQ ID NO: 7 - protein, 8 aa, Artificial Sequence
  HCDR1
GYSFTSYW

SEQ ID NO: 8 - protein, 8 aa, Artificial Sequence
  HCDR2
IYPGNSDT

SEQ ID NO: 9 - protein, 13 aa, Artificial Sequence
  HCDR3
TTEGLMNGLHFDM

SEQ ID NO: 10 - protein, 11 aa, Artificial Sequence
  LCDR1
QSLLHSLGDNY

SEQ ID NO: 11 - protein, 3 aa, Artificial Sequence
  LCDR2
LGS

SEQ ID NO: 12 - protein, 10 aa, Artificial Sequence
  LCDR3
MQSLQTPPYT

SEQ ID NO: 13 - protein, 8 aa, Artificial Sequence
  HCDR1
GFTFSSYS

SEQ ID NO: 14 - protein, 8 aa, Artificial Sequence
  HCDR2
ISASDGAT

SEQ ID NO: 15 - protein, 16 aa, Artificial Sequence
  HCDR3
AKILAGYSGPMGGMDV

SEQ ID NO: 16 - protein, 6 aa, Artificial Sequence
  LCDR1
RDISNY

SEQ ID NO: 17 - protein, 3 aa, Artificial Sequence
  LCDR2
GAS

SEQ ID NO: 18 - protein, 9 aa, Artificial Sequence
  LCDR3
QQYYSYPLT

SEQ ID NO: 19 - protein, 8 aa, Artificial Sequence
  HCDR1
GFAFGRYE

SEQ ID NO: 20 - protein, 8 aa, Artificial Sequence
  HCDR2
IDTGGGAK

SEQ ID NO: 21 - protein, 13 aa, Artificial Sequence
  HCDR3
TTEGLMNGLHFDM

SEQ ID NO: 22 - protein, 6 aa, Artificial Sequence
  LCDR1
QAISTW

SEQ ID NO: 23 - protein, 3 aa, Artificial Sequence
  LCDR2
TAS

SEQ ID NO: 24 - protein, 9 aa, Artificial Sequence
  LCDR3
QQLNSYPYT

SEQ ID NO: 25 - protein, 8 aa, Artificial Sequence
  HCDR1
GFTFDDCA

SEQ ID NO: 26 - protein, 8 aa, Artificial Sequence
  HCDR2
ISGNSKNV

SEQ ID NO: 27 - protein, 11 aa, Artificial Sequence
  HCDR3
ARDPAYSQFDY

SEQ ID NO: 28 - protein, 8 aa, Artificial Sequence
  LCDR1
SSNVGGYP

SEQ ID NO: 29 - protein, 3 aa, Artificial Sequence
  LCDR2
TDY

SEQ ID NO: 30 - protein, 11 aa, Artificial Sequence
  LCDR3
ATWDDNLNGYV

SEQ ID NO: 31 - protein, 123 aa, Artificial Sequence
  V12S VH
QVQLVESGGGLSKPGGSLRLSCAASGFTFSSYSMNWVRQAPGKGLEWVSSISASDGATYYADSVRGRFTISRDNSRSTLYLQMNSLRAEDTAVYYCAKTLAGYSGPMGGMDVWGQGTTVTVSS

SEQ ID NO: 32 - protein, 108 aa, Artificial Sequence
  V12S VL
DIQMTQSPSSLSASVGDRVTITCRASRDISNYLAWYQQKPGKAPKSLIYGASNLQSGVSSQFSGSGSGTDFTLTINSLQPEDSATYYCQQYYSYPLTFGGGTKVDIKR

SEQ ID NO: 33 - protein, 123 aa, Artificial Sequence
  N35T VH
QVQLVESGGGLVKPGGSLRLSCAASGFTFSSYSMTWVRQAPGKGLEWVSSISASDGATYYADSVRGRFTISRDNSRSTLYLQMNSLRAEDTAVYYCAKTLAGYSGPMGGMDVWGQGTTVTVSS

SEQ ID NO: 34 - protein, 123 aa, Artificial Sequence
  N76S VH
QVQLVESGGGLVKPGGSLRLSCAASGFTFSSYSMNWVRQAPGKGLEWVSSISASDGATYYADSVRGRFTISRDNSRSTLYLQMNSLRAEDTAVYYCAKTLAGYSGPMGGMDVWGQGTTVTVSS

SEQ ID NO: 35 - protein, 108 aa, Artificial Sequence
  N76S VL
DIQMTQSPSSLSASVGDRVTITCRASRDISNYLAWYQQKPGKAPKSLIYGASNLQSGVSSQFSGSGSGTDFTLTISSLQPEDSATYYCQQYYSYPLTFGGGTKVDIKR

SEQ ID NO: 36 - protein, 123 aa, Artificial Sequence
  V12S-N35T VH
QVQLVESGGGLSKPGGSLRLSCAASGFTFSSYSMTWVRQAPGKGLEWVSSISASDGATYYADSVRGRFTISRDNSRSTLYLQMNSLRAEDTAVYYCAKTLAGYSGPMGGMDVWGQGTTVTVSS

SEQ ID NO: 37 - DNA, 369 bp, Artificial Sequence
  V12S
caggtgcagctggtagagtctgggggaggcctgtccaagcctggggggtccctgagactctcctgtgcagcctctggattcaccttcagtagctatagcatgaactgggtccgccaggctccagggaaggggctggagtgggtctcatccattagtgctagtgatggtgccacatactacgcagactccgtgaggggccggttcaccatctccagagacaattccaggagcacactgtatctgcaaatgaacagtctgagagccgaggacacggccgtgtattactgtgcgaaaactctcgcgggatatagtggcccaatgggtggcatggacgtctggggccaagggaccacggtcaccgtctcctca

SEQ ID NO: 38 - DNA, 324 bp, Artificial Sequence
  VL-O4
gacatccagatgacccagtctccatcctcactgtctgcatctgtaggagacagagtcaccatcacttgtcgggcgagtcgggacattagcaactatttagcctggtatcagcagaaaccagggaaagcccctaagtccctgatctatggagcatccaatttacaaagtggggtctcatcacagttcagcggcagtggatccgggacagatttcaccctcaccatcaacagcctgcagcctgaagattctgcaacttattactgtcaacagtactatagttacccgctcacttttggcggagggaccaaggtggatatcaaacgt

SEQ ID NO: 39 - DNA, 369 bp, Artificial Sequence
  N35T
caggtgcagctggtagagtctgggggaggcctggtcaagcctggggggtccctgagactctcctgtgcagcctctggattcaccttcagtagctatagcatgacctgggtccgccaggctccagggaaggggctggagtgggtctcatccattagtgctagtgatggtgccacatactacgcagactccgtgaggggccggttcaccatctccagagacaattccaggagcacactgtatctgcaaatgaacagtctgagagccgaggacacggccgtgtattactgtgcgaaaactctcgcgggatatagtggcccaatgggtggcatggacgtctggggccaagggaccacggtcaccgtctcctca

SEQ ID NO: 40 - DNA, 369 bp, Artificial Sequence
  VH-O4
caggtgcagctggtagagtctgggggaggcctggtcaagcctggggggtccctgagactctcctgtgcagcctctggattcaccttcagtagctatagcatgaactgggtccgccaggctccagggaaggggctggagtgggtctcatccattagtgctagtgatggtgccacatactacgcagactccgtgaggggccggttcaccatctccagagacaattccaggagcacactgtatctgcaaatgaacagtctgagagccgaggacacggccgtgtattactgtgcgaaaactctcgcgggatatagtggcccaatgggtggcatggacgtctggggccaagggaccacggtcaccgtctcctca

SEQ ID NO: 41 - DNA, 324 bp, Artificial Sequence
  N76S
gacatccagatgacccagtctccatcctcactgtctgcatctgtaggagacagagtcaccatcacttgtcgggcgagtcgggacattagcaactatttagcctggtatcagcagaaaccagggaaagcccctaagtccctgatctatggagcatccaatttacaaagtggggtctcatcacagttcagcggcagtggatccgggacagatttcaccctcaccatcagcagcctgcagcctgaagattctgcaacttattactgtcaacagtactatagttacccgctcacttttggcggagggaccaaggtggatatcaaacgt

SEQ ID NO: 42 - DNA, 369 bp, Artificial Sequence
  V12S/N35T
caggtgcagctggtagagtctgggggaggcctgtccaagcctggggggtccctgagactctcctgtgcagcctctggattcaccttcagtagctatagcatgacctgggtccgccaggctccagggaaggggctggagtgggtctcatccattagtgctagtgatggtgccacatactacgcagactccgtgaggggccggttcaccatctccagagacaattccaggagcacactgtatctgcaaatgaacagtctgagagccgaggacacggccgtgtattactgtgcgaaaactctcgcgggatatagtggcccaatgggtggcatggacgtctggggccaagggaccacggtcaccgtctcctca

SEQ ID NO: 43 - protein, 16 aa, Artificial Sequence
  Synthetic CDR3
AKTLAGYSGPMGGMDV

SEQ ID NO: 44 - protein, 16 aa, Artificial Sequence
  Synthetic CDR3
AKILVGYSGPMGGMDV

SEQ ID NO: 45 - protein, 16 aa, Artificial Sequence
  Synthetic CDR3
AKSLASYSGPMGGMDV

SEQ ID NO: 46 - protein, 123 aa, Artificial Sequence
  L11T
QVQLVESGGGTVKPGGSLRLSCAASGFTFSSYSMNWVRQAPGKGLEWVSSISASDGATYYADSVRGRFTISRDNSRSTLYLQMNSLRAEDTAVYYCAKTLAGYSGPMGGMDVWGQGTTVTVSS

SEQ ID NO: 47 - DNA, 369 bp, Artificial Sequence
  L11T
caggtgcagctggtagagtctgggggaggcacggtcaagcctggggggtccctgagactctcctgtgcagcctctggattcaccttcagtagctatagcatgaactgggtccgccaggctccagggaaggggctggagtgggtctcatccattagtgctagtgatggtgccacatactacgcagactccgtgaggggccggttcaccatctccagagacaattccaggagcacactgtatctgcaaatgaacagtctgagagccgaggacacggccgtgtattactgtgcgaaaactctcgcgggatatagtggcccaatgggtggcatggacgtctggggccaagggaccacggtcaccgtctcctca

SEQ ID NO: 48 - protein, 123 aa, Artificial Sequence
  V93S
QVQLVESGGGLVKPGGSLRLSCAASGFTFSSYSMNWVRQAPGKGLEWVSSISASDGATYYADSVRGRFTISRDNSRSTLYLQMNSLRAEDTASYYCAKTLAGYSGPMGGMDVWGQGTTVTVSS

SEQ ID NO: 49 - DNA, 369 bp, Artificial Sequence
  V93S
caggtgcagctggtagagtctgggggaggcctggtcaagcctggggggtccctgagactctcctgtgcagcctctggattcaccttcagtagctatagcatgaactgggtccgccaggctccagggaaggggctggagtgggtctcatccattagtgctagtgatggtgccacatactacgcagactccgtgaggggccggttcaccatctccagagacaattccaggagcacactgtatctgcaaatgaacagtctgagagccgaggacacggcctcgtattactgtgcgaaaactctcgcgggatatagtggcccaatgggtggcatggacgtctggggccaagggaccacggtcaccgtctcctca

SEQ ID NO: 50 - protein, 108 aa, Artificial Sequence
  Q61R
DIQMTQSPSSLSASVGDRVTITCRASRDISNYLAWYQQKPGKAPKSLIYGASNLQSGVSSRFSGSGSGTDFTLTINSLQPEDSATYYCQQYYSYPLTFGGGTKVDIKR

SEQ ID NO: 51 - DNA, 324 bp, Artificial Sequence
  Q61R
gacatccagatgacccagtctccatcctcactgtctgcatctgtaggagacagagtcaccatcacttgtcgggcgagtcgggacattagcaactatttagcctggtatcagcagaaaccagggaaagcccctaagtccctgatctatggagcatccaatttacaaagtggggtctcatcacggttcagcggcagtggatccgggacagatttcaccctcaccatcaacagcctgcagcctgaagattctgcaacttattactgtcaacagtactatagttacccgctcacttttggcggagggaccaaggtggatatcaaacgt